European Patent Application EP 4 692 356 A1, published February 11, 2026. Title: Promoters suitable for driving gene expression in hydrogen bacteria. Applicant: Logomix, Inc. The sequence listing filed with the application follows.

SEQUENCE LISTING (19 sequences)

SEQ ID NO: 1 - DNA, 300 bp, Ralstonia eutropha H16
  source 1..300: mol_type = genomic DNA
tgccgcggcaagcgccggcgtcgacccgcgccagtgcgtctatgtgggcgatgacctgcgcgacatccaggccggcaaggccgccggcatgatcaccgtcacagccgcctatggctattgcggcgacgccgagccgcccgagacctggggcgccgaccacctgattcgccacccggccgagctgatcccgctgctgttgcccgccgtggtcgcctgattgtgtcgcaggggtatcctggccgttcccggaactccccgcgacagcttgcgtccaaccgggtacaatccagcttcctcact

SEQ ID NO: 2 - DNA, 300 bp, Ralstonia eutropha H16
  source 1..300: mol_type = genomic DNA
tttgtcggccgtccgtcacctgaagcgactgcttcaggggaaacgcagcccgactaattcggctgaggtaggcctttcgtatctgctaatccccgtttttgcaccaaaacggggattttccctcccattcctgttgctcccccacaacaaaaaccgccagtaagcatggtttacgccgaaaaagccttctgacggccgggggggctggcacataatacgcagcagacgtgaatgtaaatgcgtcgcccaagtacttgggcaaccaagatttcccaatcagttgacaaggaaagtgtcgat

SEQ ID NO: 3 - DNA, 300 bp, Ralstonia eutropha H16
  source 1..300: mol_type = genomic DNA
tactcgaaaaactggtgcagccgtacaagtcggtcactgcccatgcatgggtgctgccgctggcgccgcagcaggcggcaggcccgtggctggacgtcatgctggcgcaatcccttgccgctgcggcccaggctggcgcgctgcgcggcgggcgcagttttgcgccgctgccggtgatgggtattccgggctggtgcgacgataacgccgaacctggcttctacgccgatacctctgtgttccgcccaggacggcgcgccgactgaaggcgccgccaatcggtgttagactgcgggccgc

SEQ ID NO: 4 - DNA, 300 bp, Ralstonia eutropha H16
  source 1..300: mol_type = genomic DNA
acgctcaacagcaccccattgctggcaatgtgccggttccgagaatagttcgtataacctccgcccattgtgaaggattactttttgttacattcgggggagtccctggtagggttatttcaacgctattaaaaatattgaaattattcctcttcggccctaaggaaccttttgatagcatgcacgccgctgctgccggataaccgttcgcatcagtgttttcctttacatatggcttccatatgaggcgcctttcatatggcgcaaccgtttctgtgcattcccatggaaggagtcgtt

SEQ ID NO: 5 - DNA, 300 bp, Ralstonia eutropha H16
  source 1..300: mol_type = genomic DNA
gccagctgtccgatatctcctcatttctggccgtgcgccggctcaacgggcggtgcgggctgatcgaatattccagggcgcggcacgtgcccgagacccgcttgcgggctcgctccggccgccaagtcaccgccaggggcggtgcgcctgcaaccaaattcattagcgtgcagcagtggtcgggccgcacgccgatgaatcgctcgctcgactggggccgcgctgctgtagtgcgcctcgggtcggtcgggtcgccaacttaggtcattcgatattcactctctagtgaaggagttatcc

SEQ ID NO: 6 - DNA, 300 bp, Ralstonia eutropha H16
  source 1..300: mol_type = genomic DNA
cgtgaccaggcagcaaacggtagcgccgcagcacgcgcatcgctgcgcgcacaggcaccgaagagcctgccgcgaacgccaaaacgggggtacgtaggccgtattcgcgtttccactgaggcaaagccgcgacaaaacccggggttttcacggggttttacgtttcgaatgcacgaaaaccccttgacttacggtactttccgctatgattcagtgggcgtcgagcagacgattgcgcaacgctgagaagcaatgcgaaacacctgccgacacccatctgttcaacttacgaatatcgat

SEQ ID NO: 7 - DNA, 300 bp, Ralstonia eutropha H16
  source 1..300: mol_type = genomic DNA
cgttatggtgcggcgccccatttgtgggaatctatcctatgctgctggtttgccccacgcgcgggccggtctggcgttgccgcgctgcgggacggcccggcaaagccggcttctggcaagcgggaaaagcgtggaaaattgcccgctaaccggcctcaatcaaggatttgcgggtttttttgtcgcattggtgccactggggattgctctacgcgcgacgggcagattagactgcgccgatcgatggctttgccgcgaggcacgcacatcggtgacgacgaccaacaagggaaatcagcc

SEQ ID NO: 8 - DNA, 300 bp, Ralstonia eutropha H16
  source 1..300: mol_type = genomic DNA
attttggctggcattgcggccgtatgaccgcaatgccaggttgcaggccggttcccggccggtctgcctgctctttgacaacctgtggacccgggcgtgccgggtcgtttcaaacgcgcgtcttaacccctttgggtcattgctatcacccgtaggaggggtatggttgagacattccatgtcttaaaaagaaagcgcagcaagcgtgaaaagtcgataaaatagcgggccacagagcaccgtgataatcgaacgggggaagcgtgatcgcggcaacagatcacttcgggagtggaaatc

SEQ ID NO: 9 - DNA, 300 bp, Ralstonia eutropha H16
  source 1..300: mol_type = genomic DNA
ccgttttccaaatttacaaaatatatgttgccaacgcagagagcagaggccgccatttggcagccggaaacgagccgtaccgtaaaattgcttgaaaaacagcccgggatgtgcctaaagtatctatagtgcgcattacgccgcacatgacaccgcaatccaaagtggttatgatgcgcgctacagtcgagtcaagtcgtgtcaacctcgtcggcttccgttcggtatctacgagaactcaacgtgcttgaacggttgtttgcgttgtgtacaagaacttgcttcgaaaaggaaattcct

SEQ ID NO: 10 - DNA, 300 bp, Ralstonia eutropha H16
  source 1..300: mol_type = genomic DNA
cttgcgcacacctcccgaggccctcgctgaaacccggaatccctgatgccacaaggctttgcgggcgacacaagacctatgttgcacaaacaccacaggcccaaaacccatgcggcgaatcgaatatatttacttcttaggaaacgacccttgtggcacaattccccagcgaagagccagacattgttcgaagtggagcatccaccacatcgagaatgttatactccgaagaatgtatgacttgttttcgtccatttgctcgcagtaaccctgcggtgatctcatcctgagaggagaaat

SEQ ID NO: 11 - DNA, 300 bp, Ralstonia eutropha H16
  source 1..300: mol_type = genomic DNA
tgaactgaagctgaagtagaaaacgctaatatctcctatcggaacctctcatcatgattaggcgcttagcctgattgacacgccgggaaaattcggcagaatgattcccacttgtgcagcgcccatgcggtgtgtcttttggtgttgtcgttccgtgacgttttcggttgtcacgacagcgacatatcgaagtcatatggaatgcgctggcggggaacataaaaaggatccgctgggtgcgttgcacacggtgtataacgagcgttttcgctcattttgaaattcaaggttgagatagat

SEQ ID NO: 12 - DNA, 300 bp, Ralstonia eutropha H16
  source 1..300: mol_type = genomic DNA
tctcctgatttcggggtggaaccagagtatccggattgatatccaacccaaacgaatataaagtcactacaaaatcactcgaagtcataaagacattttgtgacattgatcacgcgtgctttccggcatgcttgcgataccaggcactgcagagtcgcgcttgctggcgtgtagccttgaaaccaccgccgcccgccacatatgctaagtatcagaccgacaaatgccgttagcctcggagcgtagaaaatgtcagaatccgcacaaaccgaaccaaccgcccgcaaacaggagaaactg

SEQ ID NO: 13 - DNA, 300 bp, Ralstonia eutropha H16
  source 1..300: mol_type = genomic DNA
cctgctggcagtggggaatccgccaacttgacagtatcctgctttgccagaagaatcgttcgcacacctgccgacggccaacgagccaaagcaacagccgagacaggtgatccgtgagcagggaggccacggccgccgcggcggcgagtcagcatcgagactgtccgccacgcgattgcacctcgccgcgcgtcatcgccggccgcgcctcaggacgcggcaggtcatggcgccgcagtccgtgccgtctggccggcaaggcttccccgctttgaaatctgctatttcgtgggggagtat

SEQ ID NO: 14 - DNA, 300 bp, Ralstonia eutropha H16
  source 1..300: mol_type = genomic DNA
gttggaagcggatgcggcagacccggaaccgggacgcgccggtagccgcacttcgcggggctggcgctatggtatcgcaatgccggccttgcgcagcacctcagcgatgtcgtcaccggcgtcgccagcagatgccatacattcgttaaatttgtcattttggaaatttcctggcagacagaattaaaaaacgctgaatggcatttctgcgttggatgcaatacattccatacattgaaaatccagtgcgagcgcatacccgcccccggccgcaccttgcagcaatcctggagtgtgtcc

SEQ ID NO: 15 - DNA, 300 bp, Ralstonia eutropha H16
  source 1..300: mol_type = genomic DNA
cgcgaggggtcatgaccggctgccacctggcagccggtttttttatggctgccagttgaaaatgtgccatcagtcacccacatctgccccagaatcgttgcatttgatccggcgcagtacgcaggcaacgccatcggtattcaatacttgtagaagaaactttcactttgcggacaagcgctgactcggtacattaaccgggtgttccgccacatgtgcccagccgccaccggccaggctcggccccaaaaccggattcgcgcaggcgctgcgcgaccgtcaatcgcgaggataagcaag

SEQ ID NO: 16 - DNA, 300 bp, Ralstonia eutropha H16
  source 1..300: mol_type = genomic DNA
aaaatctgctggctcatcaggggctccggtagtcgtgtcagagggggctgcgccgggcgcagacaagcagtctaggcgctaaaggccgggggcgtgcgtattttcattgtccttaaatgcgggcaaaacgggcgatgcccagcccaataccggctgcatcgtgggctgtgcgaccgtcaattcaggccagcaaacaatcagtccgtgcaatctccgttattttttgtaaaatttttttaggtgaaccgacaccacacttctagtaccatgcagcggcctatttgcagaaaggggatataa

SEQ ID NO: 17 - DNA, 300 bp, Ralstonia insidiosa
  source 1..300: mol_type = genomic DNA
cgctgtacaagatcgacatgatcatggacggcgacatggatgagctgctgtcggcactggcttcggaacaccaggctgatcagcttgctgcacttggcgaagagtcgtaagcaccacaaaatgtcgtgcaaccggccttccgccccgaacaccgcgtaaagtcgccgatatctttgtatttcttgtaaatgcttgaaacagcactggtaggggtaaggcggctgtctataatcgatttcgaccggcaaacggagaatggtgccgggtagtcactcccgagaacatacctaggacgaaatc

SEQ ID NO: 18 - DNA, 300 bp, Ralstonia eutropha H16
  source 1..300: mol_type = genomic DNA
aatacgtgctaacccacccgaacgcgaagatcccgcaggtacctgctggttcgcgatctgcgcttcggccaagtacttctgggcagtcttgaaggaggctcaatgattcagtgtgcattcaagattgtgatgaaagccgtagggaagaattgcgcatcgggtcaaaggccgggttgtcgtgacgctccccaggcgctcgcgccgcattgcggcccgtgcctgcgacggccctcgacgctggcgatcggagttgcggtaagctgctgcgccatccctcatggcgcctcgatcgccggcggc

SEQ ID NO: 19 - DNA, 300 bp, Ralstonia eutropha H16
  source 1..300: mol_type = genomic DNA
aggctggttcttatcagttcaaaccgaggggactttgcacccgaatcacgcgcattgttttacggcgctccctttaatgcagttctcgctgcccttaccgcatggagcctcactgtggcgcggcggtggtactcagtcgctgtcatactttctcgctcagcttttttggtcatgattcggagccgccaagcgaatcattggactgctcattacccagaaggttaaagtttttatgccctgaagatcaaattggctctaaactacctatctggatctctcgatcggaaaggaaaccagaag